European Patent Specification EP 3 934 689 B1, published April 23, 2025. Title: METHODS OF TREATING AL AMYLOIDOSIS. Applicant: PROTHENA BIOSCIENCES LIMITED KINNEY, Gene KARP, Carol ZAGO, Wanger M TRIPURANENI, Radhika M. The sequence listing filed with the application follows.

SEQUENCE LISTING (23 sequences)

SEQ ID NO: 1 - protein, 112 aa, Artificial Sequence
  Synthetic peptide
DVVMTQSPLSLPVTPGEPASISCRSSQSLVHSTGNTYLHWYLQKPGQSPQLLIYKVSNRFSGVPDRFSGSGSGTDFTLKISRVEAEDVGVYYCSQSTHVPFTFGGGTKVEIK

SEQ ID NO: 2 - protein, 119 aa, Artificial Sequence
  Synthetic peptide
EVQLVESGGGLVQPGGSLRLSCAASGFTFNTYAMYWIRQAPGKGLEWVARIRSKSNNYAIYYADSVKDRFTISRDDSKNSLYLQMNSLKTEDTAVYYCARPYSDSFAYWGQGTLVTVSS

SEQ ID NO: 3 - protein, 16 aa, Artificial Sequence
  Synthetic peptide
RSSQSLVHSTGNTYLH

SEQ ID NO: 4 - protein, 7 aa, Artificial Sequence
  Synthetic peptide
KVSNRFS

SEQ ID NO: 5 - protein, 9 aa, Artificial Sequence
  Synthetic peptide
SQSTHVPFT

SEQ ID NO: 6 - protein, 10 aa, Artificial Sequence
  Synthetic peptide
GFTFNTYAMY

SEQ ID NO: 7 - protein, 19 aa, Artificial Sequence
  Synthetic peptide
RIRSKSNNYAIYYADSVKD

SEQ ID NO: 8 - protein, 8 aa, Artificial Sequence
  Synthetic peptide
PYSDSFAY

SEQ ID NO: 9 - protein, 16 aa, Artificial Sequence
  Synthetic peptide
RSSLSLVHSTGNTYLH

SEQ ID NO: 10 - protein, 219 aa, Artificial Sequence
  Synthetic peptide
DVVMTQSPLSLPVTPGEPASISCRSSQSLVHSTGNTYLHWYLQKPGQSPQLLIYKVSNRFSGVPDRFSGSGSGTDFTLKISRVEAEDVGVYYCSQSTHVPFTFGGGTKVEIKRTVAAPSVFIFPPSDEQLKSGTASVVCLLNNFYPREAKVQWKVDNALQSGNSQESVTEQDSKDSTYSLSSTLTLSKADYEKHKVYACEVTHQGLSSPVTKSFNRGEC

SEQ ID NO: 11 - protein, 449 aa, Artificial Sequence
  Synthetic peptide
EVQLVESGGGLVQPGGSLRLSCAASGFTFNTYAMYWIRQAPGKGLEWVARIRSKSNNYAIYYADSVKDRFTISRDDSKNSLYLQMNSLKTEDTAVYYCARPYSDSFAYWGQGTLVTVSSASTKGPSVFPLAPSSKSTSGGTAALGCLVKDYFPEPVTVSWNSGALTSGVHTFPAVLQSSGLYSLSSVVTVPSSSLGTQTYICNVNHKPSNTKVDKRVEPKSCDKTHTCPPCPAPELLGGPSVFLFPPKPKDTLMISRTPEVTCVVVDVSHEDPEVKFNWYVDGVEVHNAKTKPREEQYNSTYRVVSVLTVLHQDWLNGKEYKCKVSNKALPAPIEKTISKAKGQPREPQVYTLPPSRDELTKNQVSLTCLVKGFYPSDIAVEWESNGQPENNYKTTPPVLDSDGSFFLYSKLTVDKSRWQQGNVFSCSVMHEALHNHYTQKSLSLSPGK

SEQ ID NO: 12 - protein, 449 aa, Artificial Sequence
  Synthetic peptide
EVQLVESGGGLVQPGGSLRLSCAASGFTFNTYAMYWIRQAPGKGLEWVARIRSKSNNYAIYYADSVKDRFTISRDDSKNSLYLQMNSLKTEDTAVYYCARPYSDSFAYWGQGTLVTVSSASTKGPSVFPLAPSSKSTSGGTAALGCLVKDYFPEPVTVSWNSGALTSGVHTFPAVLQSSGLYSLSSVVTVPSSSLGTQTYICNVNHKPSNTKVDKRVEPKSCDKTHTCPPCPAPELLGGPSVFLFPPKPKDTLMISRTPEVTCVVVDVSHEDPEVKFNWYVDGVEVHNAKTKPREEQYNSTYRVVSVLTVLHQDWLNGKEYKCKVSNKALPAPIEKTISKAKGQPREPQVYTLPPSREEMTKNQVSLTCLVKGFYPSDIAVEWESNGQPENNYKTTPPVLDSDGSFFLYSKLTVDKSRWQQGNVFSCSVMHEALHNHYTQKSLSLSPGK

SEQ ID NO: 13 - protein, 445 aa, Artificial Sequence
  Synthetic peptide
EVQLVESGGGLVQPGGSLRLSCAASGFTFNTYAMYWIRQAPGKGLEWVARIRSKSNNYAIYYADSVKDRFTISRDDSKNSLYLQMNSLKTEDTAVYYCARPYSDSFAYWGQGTLVTVSSASTKGPSVFPLAPCSRSTSESTAALGCLVKDYFPEPVTVSWNSGALTSGVHTFPAVLQSSGLYSLSSVVTVPSSNFGTQTYTCNVDHKPSNTKVDKTVERKCCVECPPCPAPPVAGPSVFLFPPKPKDTLMISRTPEVTCVVVDVSHEDPEVQFNWYVDGVEVHNAKTKPREEQFNSTFRVVSVLTVVHQDWLNGKEYKCKVSNKGLPAPIEKTISKTKGQPREPQVYTLPPSREEMTKNQVSLTCLVKGFYPSDIAVEWESNGQPENNYKTTPPMLDSDGSFFLYSKLTVDKSRWQQGNVFSCSVMHEALHNHYTQKSLSLSPGK

SEQ ID NO: 14 - protein, 112 aa, Artificial Sequence
  Synthetic peptide
DVVMTQTPLSLPVSLGDQASISCRSSQSLVHRNGNTYLHWYLQKPGQSPKLLIYKVSNRFSGVPDRFSGSGSGTDFTLKISRVEAEDLGLYFCFQTTYVPNTFGGGTKLEIK

SEQ ID NO: 15 - protein, 111 aa, Artificial Sequence
  Synthetic peptide
QVQLKESGPGLVAPSQSLSITCTVSGFSLSSYGVSWVRQPPGKGLEWLGVIWGDGSTNYKPNLMSRLSISKDISKSQVLFKLNSLQTDDTATYYCVTLDYWGQGTSVTVSS

SEQ ID NO: 16 - protein, 16 aa, Artificial Sequence
  Synthetic peptide
RSSQSLVHRNGNYTLH

SEQ ID NO: 17 - protein, 7 aa, Artificial Sequence
  Synthetic peptide
LVSNRFS

SEQ ID NO: 18 - protein, 9 aa, Artificial Sequence
  Synthetic peptide
FNTTYVPNT

SEQ ID NO: 19 - protein, 6 aa, Artificial Sequence
  Synthetic peptide
SYGVSW

SEQ ID NO: 20 - protein, 21 aa, Artificial Sequence
  Synthetic peptide
VIWGDGSTNYHPNLMSRLSIS

SEQ ID NO: 21 - protein, 3 aa, Artificial Sequence
  Synthetic peptide
LDY

SEQ ID NO: 22 - DNA, 336 bp, Artificial Sequence
  11-1F4 monoclonal antibody variable light
gatgttgtgatgacccaaactccactctccctgcctgtcagtcttggagatcaagcctccatctcttgcagatctagtcagagccttgtacatagaaatggaaacacctatttacattggtacctgcagaagccaggccagtctccaaagctcctgatctacaaagtttccaaccgattttctggggtcccagacaggttcagtggcagtggatcagggacagatttcacactcaagatcagcagagtggaggctgaggatttgggactttatttctgttttcaaactacatatgttccgaacacgttcggaggggggaccaagctggaaataaaa

SEQ ID NO: 23 - DNA, 333 bp, Artificial Sequence
  11-1F4 monoclonal antibody variable heavy
caggtgcagctgaaggagtcaggacctggcctggtggcgccctcacagagcctgtccatcacatgcactgtctcagggttctcattaagcagctatggtgtaagctgggttcgccagcctccaggaaagggtctggagtggctgggagtaatatggggtgacgggagcacaaattatcatccaaatctcatgtccagactgagtatcagcaaggatatttccaagagccaagttctcttcaaactgaatagtctgcaaactgatgacacagccacgtactactgtgtcaccttcgactactggggtcaaggaacctcagtcaccgtctcctca